European Patent Application EP 4 534 692 A2, published April 9, 2025. Title: METHODS AND SYSTEMS FOR GENERATION AND ERROR-CORRECTION OF UNIQUE MOLECULAR INDEX SETS WITH HETEROGENEOUS MOLECULAR LENGTHS. Applicant: ILLUMINA, INC. Application EP. The sequence listing filed with the application follows.

SEQUENCE LISTING (2 sequences)

SEQ ID NO: 1 - skipped

SEQ ID NO: 2 - DNA, 16 bp, synthetic construct
  misc_feature 12..16: note = n is a, c, g, or t
  source 1..16: mol_type = other DNA
ttggcatgactnnnnn